European Patent Application EP 4 252 759 A2, published October 4, 2023. Title: T CELL RECEPTORS TARGETING PIK3CA MUTATIONS AND USES THEREOF. Applicant: MEMORIAL SLOAN-KETTERING CANCER CENTER. Application WO PCT/US2019/031749, filed May 10, 2019. The sequence listing filed with the application follows.

SEQUENCE LISTING (131 sequences)

SEQ ID NO: 1 - protein, 6 aa, synthetic construct
  REGION 1..6: note = Description of Artificial Sequence: Synthetic peptide
DSAIYN

SEQ ID NO: 2 - protein, 7 aa, synthetic construct
  REGION 1..7: note = Description of Artificial Sequence: Synthetic peptide
IQSSQRE

SEQ ID NO: 3 - protein, 13 aa, synthetic construct
  REGION 1..13: note = Description of Artificial Sequence: Synthetic peptide
CAVKGSDDYKLSF

SEQ ID NO: 4 - protein, 5 aa, synthetic construct
  REGION 1..5: note = Description of Artificial Sequence: Synthetic peptide
KGHSH

SEQ ID NO: 5 - protein, 5 aa, synthetic construct
  REGION 1..5: note = Description of Artificial Sequence: Synthetic peptide
KGHSH

SEQ ID NO: 6 - protein, 19 aa, synthetic construct
  REGION 1..19: note = Description of Artificial Sequence: Synthetic peptide
CASSPVNLAGVSRADTQYF

SEQ ID NO: 7 - protein, 131 aa, synthetic construct
  REGION 1..131: note = Description of Artificial Sequence: Synthetic polypeptide
METLLGLLILWLQLQWVSSKQEVTQIPAALSVPEGENLVLNCSFTDSAIYNLQWFRQDPGKGLTSLLLIQSSQREQTSGRLNASLDKSSGRSTLYIAASQPGDSATYLCAVKGSDDYKLSFGAGTTVTVRA

SEQ ID NO: 8 - protein, 138 aa, synthetic construct
  REGION 1..138: note = Description of Artificial Sequence: Synthetic polypeptide
MDTRVLCCAVICLLGAGLSNAGVMQNPRHLVRRRGQEARLRCSPMKGHSHVYWYRQLPEEGLKFMVYLQKENIIDESGMPKERFSAEFPKEGPSILRIQQVVRGDSAAYFCASSPVNLAGVSRADTQYFGPGTRLTVL

SEQ ID NO: 9 - protein, 268 aa, synthetic construct
  REGION 1..268: note = Description of Artificial Sequence: Synthetic polypeptide
METLLGLLILWLQLQWVSSKQEVTQIPAALSVPEGENLVLNCSFTDSAIYNLQWFRQDPGKGLTSLLLIQSSQREQTSGRLNASLDKSSGRSTLYIAASQPGDSATYLCAVKGSDDYKLSFGAGTTVTVRANIQNPEPAVYQLKDPRSQDSTLCLFTDFDSQINVPKTMESGTFITDKCVLDMKAMDSKSNGAIAWSNQTSFTCQDIFKETNATYPSSDVPCDATLTEKSFETDMNLNFQNLLVIVLRILLLKVAGFNLLMTLRLWSS

SEQ ID NO: 10 - protein, 311 aa, synthetic construct
  REGION 1..311: note = Description of Artificial Sequence: Synthetic polypeptide
MDTRVLCCAVICLLGAGLSNAGVMQNPRHLVRRRGQEARLRCSPMKGHSHVYWYRQLPEEGLKFMVYLQKENIIDESGMPKERFSAEFPKEGPSILRIQQVVRGDSAAYFCASSPVNLAGVSRADTQYFGPGTRLTVLEDLRNVTPPKVSLFEPSKAEIANKQKATLVCLARGFFPDHVELSWWVNGKEVHSGVCTDPQAYKESNYSYCLSSRLRVSATFWHNPRNHFRCQVQFHGLSEEDKWPEGSPKPVTQNISAEAWGRADCGITSASYQQGVLSATILYEILLGKATLYAVLVSTLVVMAMVKRKNS

SEQ ID NO: 11 - protein, 6 aa, synthetic construct
  REGION 1..6: note = Description of Artificial Sequence: Synthetic peptide
TSGFNG

SEQ ID NO: 12 - protein, 6 aa, synthetic construct
  REGION 1..6: note = Description of Artificial Sequence: Synthetic peptide
NVLDGL

SEQ ID NO: 13 - protein, 11 aa, synthetic construct
  REGION 1..11: note = Description of Artificial Sequence: Synthetic peptide
CAVTSWGKLQF

SEQ ID NO: 14 - protein, 5 aa, synthetic construct
  REGION 1..5: note = Description of Artificial Sequence: Synthetic peptide
SGHTA

SEQ ID NO: 15 - protein, 6 aa, synthetic construct
  REGION 1..6: note = Description of Artificial Sequence: Synthetic peptide
FQGNSA

SEQ ID NO: 16 - protein, 13 aa, synthetic construct
  REGION 1..13: note = Description of Artificial Sequence: Synthetic peptide
CASSPRGYQPQHF

SEQ ID NO: 17 - protein, 129 aa, synthetic construct
  REGION 1..129: note = Description of Artificial Sequence: Synthetic polypeptide
MWGVFLLYVSMKMGGTTGQNIDQPTEMTATEGAIVQINCTYQTSGFNGLFWYQQHAGEAPTFLSYNVLDGLEEKGRFSSFLSRSKGYSYLLLKELQMKDSASYLCAVTSWGKLQFKLQFGAGTQVVVTP

SEQ ID NO: 18 - protein, 132 aa, synthetic construct
  REGION 1..132: note = Description of Artificial Sequence: Synthetic polypeptide
MGTRLLFWVAFCLLGAYHTGAGVSQSPSNKVTEKGKDVELRCDPISGHTALYWYRQRLGQGLEFLIYFQGNSAPDKSGLPSDRFSAERTGESVSTLTIQRTQQEDSAVYLCASSPRGYQPQHFGDGTRLSIL

SEQ ID NO: 19 - protein, 266 aa, synthetic construct
  REGION 1..266: note = Description of Artificial Sequence: Synthetic polypeptide
MWGVFLLYVSMKMGGTTGQNIDQPTEMTATEGAIVQINCTYQTSGFNGLFWYQQHAGEAPTFLSYNVLDGLEEKGRFSSFLSRSKGYSYLLLKELQMKDSASYLCAVTSWGKLQFKLQFGAGTQVVVTPNIQNPEPAVYQLKDPRSQDSTLCLFTDFDSQINVPKTMESGTFITDKCVLDMKAMDSKSNGAIAWSNQTSFTCQDIFKETNATYPSSDVPCDATLTEKSFETDMNLNFQNLLVIVLRILLLKVAGFNLLMTLRLWSS

SEQ ID NO: 20 - protein, 305 aa, synthetic construct
  REGION 1..305: note = Description of Artificial Sequence: Synthetic polypeptide
MGTRLLFWVAFCLLGAYHTGAGVSQSPSNKVTEKGKDVELRCDPISGHTALYWYRQRLGQGLEFLIYFQGNSAPDKSGLPSDRFSAERTGESVSTLTIQRTQQEDSAVYLCASSPRGYQPQHFGDGTRLSILEDLRNVTPPKVSLFEPSKAEIANKQKATLVCLARGFFPDHVELSWWVNGKEVHSGVCTDPQAYKESNYSYCLSSRLRVSATFWHNPRNHFRCQVQFHGLSEEDKWPEGSPKPVTQNISAEAWGRADCGITSASYQQGVLSATILYEILLGKATLYAVLVSTLVVMAMVKRKNS

SEQ ID NO: 21 - protein, 7 aa, synthetic construct
  REGION 1..7: note = Description of Artificial Sequence: Synthetic peptide
TSDQSYG

SEQ ID NO: 22 - protein, 8 aa, synthetic construct
  REGION 1..8: note = Description of Artificial Sequence: Synthetic peptide
QGSYDEQN

SEQ ID NO: 23 - protein, 15 aa, synthetic construct
  REGION 1..15: note = Description of Artificial Sequence: Synthetic peptide
CAMREVLDNTDKLIF

SEQ ID NO: 24 - protein, 5 aa, synthetic construct
  REGION 1..5: note = Description of Artificial Sequence: Synthetic peptide
KGHSH

SEQ ID NO: 25 - protein, 6 aa, synthetic construct
  REGION 1..6: note = Description of Artificial Sequence: Synthetic peptide
LQKENI

SEQ ID NO: 26 - protein, 16 aa, synthetic construct
  REGION 1..16: note = Description of Artificial Sequence: Synthetic peptide
CASSPPEAGLDTEAFF

SEQ ID NO: 27 - protein, 136 aa, synthetic construct
  REGION 1..136: note = Description of Artificial Sequence: Synthetic polypeptide
MSLSSLLKVVTASLWLGPGIAQKITQTQPGMFVQEKEAVTLDCTYDTSDQSYGLFWYKQPSSGEMIFLIYQGSYDEQNATEGRYSLNFQKARKSANLVISASQLGDSAMYFCAMREVLDNTDKLIFGTGTRLQVFP

SEQ ID NO: 28 - protein, 135 aa, synthetic construct
  REGION 1..135: note = Description of Artificial Sequence: Synthetic polypeptide
MDTRVLCCAVICLLGAGLSNAGVMQNPRHLVRRRGQEARLRCSPMKGHSHVYWYRQLPEEGLKFMVYLQKENIIDESGMPKERFSAEFPKEGPSILRIQQVVRGDSAAYFCASSPPEAGLDTEAFFGQGTRLTVV

SEQ ID NO: 29 - protein, 273 aa, synthetic construct
  REGION 1..273: note = Description of Artificial Sequence: Synthetic polypeptide
MSLSSLLKVVTASLWLGPGIAQKITQTQPGMFVQEKEAVTLDCTYDTSDQSYGLFWYKQPSSGEMIFLIYQGSYDEQNATEGRYSLNFQKARKSANLVISASQLGDSAMYFCAMREVLDNTDKLIFGTGTRLQVFPNIQNPEPAVYQLKDPRSQDSTLCLFTDFDSQINVPKTMESGTFITDKCVLDMKAMDSKSNGAIAWSNQTSFTCQDIFKETNATYPSSDVPCDATLTEKSFETDMNLNFQNLLVIVLRILLLKVAGFNLLMTLRLWSS

SEQ ID NO: 30 - protein, 308 aa, synthetic construct
  REGION 1..308: note = Description of Artificial Sequence: Synthetic polypeptide
MDTRVLCCAVICLLGAGLSNAGVMQNPRHLVRRRGQEARLRCSPMKGHSHVYWYRQLPEEGLKFMVYLQKENIIDESGMPKERFSAEFPKEGPSILRIQQVVRGDSAAYFCASSPPEAGLDTEAFFGQGTRLTVVEDLRNVTPPKVSLFEPSKAEIANKQKATLVCLARGFFPDHVELSWWVNGKEVHSGVCTDPQAYKESNYSYCLSSRLRVSATFWHNPRNHFRCQVQFHGLSEEDKWPEGSPKPVTQNISAEAWGRADCGITSASYQQGVLSATILYEILLGKATLYAVLVSTLVVMAMVKRKNS

SEQ ID NO: 31 - protein, 6 aa, synthetic construct
  REGION 1..6: note = Description of Artificial Sequence: Synthetic peptide
NSAFQY

SEQ ID NO: 32 - protein, 6 aa, synthetic construct
  REGION 1..6: note = Description of Artificial Sequence: Synthetic peptide
TYSSGN

SEQ ID NO: 33 - protein, 13 aa, synthetic construct
  REGION 1..13: note = Description of Artificial Sequence: Synthetic peptide
CAMNSGGYQKVTF

SEQ ID NO: 34 - protein, 6 aa, synthetic construct
  REGION 1..6: note = Description of Artificial Sequence: Synthetic peptide
DFQATT

SEQ ID NO: 35 - protein, 7 aa, synthetic construct
  REGION 1..7: note = Description of Artificial Sequence: Synthetic peptide
SNEGSKA

SEQ ID NO: 36 - protein, 14 aa, synthetic construct
  REGION 1..14: note = Description of Artificial Sequence: Synthetic peptide
CSAREQGPLEEQYF

SEQ ID NO: 37 - protein, 133 aa, synthetic construct
  REGION 1..133: note = Description of Artificial Sequence: Synthetic polypeptide
MMKSLRVLLVILWLQLSWVWSQQKEVEQDPGPLSVPEGAIVSLNCTYSNSAFQYFMWYRQYSRKGPELLMYTYSSGNKEDGRFTAQVDKSSKYISLFIRDSQPSDSATYLCAMNSGGYQKVTFGIGTKLQVIP

SEQ ID NO: 38 - protein, 134 aa, synthetic construct
  REGION 1..134: note = Description of Artificial Sequence: Synthetic polypeptide
MLLLLLLLGPAGSGLGAVVSQHPSRVICKSGTSVKIECRSLDFQATTMFWYRQFPKQSLMLMATSNEGSKATYEQGVEKDKFLINHASLTLSTLTVTSAHPEDSSFYICSACSAREQGPLEEQYFGPGTRLTVT

SEQ ID NO: 39 - protein, 270 aa, synthetic construct
  REGION 1..270: note = Description of Artificial Sequence: Synthetic polypeptide
MMKSLRVLLVILWLQLSWVWSQQKEVEQDPGPLSVPEGAIVSLNCTYSNSAFQYFMWYRQYSRKGPELLMYTYSSGNKEDGRFTAQVDKSSKYISLFIRDSQPSDSATYLCAMNSGGYQKVTFGIGTKLQVIPNIQNPEPAVYQLKDPRSQDSTLCLFTDFDSQINVPKTMESGTFITDKCVLDMKAMDSKSNGAIAWSNQTSFTCQDIFKETNATYPSSDVPCDATLTEKSFETDMNLNFQNLLVIVLRILLLKVAGFNLLMTLRLWSS

SEQ ID NO: 40 - protein, 307 aa, synthetic construct
  REGION 1..307: note = Description of Artificial Sequence: Synthetic polypeptide
MLLLLLLLGPAGSGLGAVVSQHPSRVICKSGTSVKIECRSLDFQATTMFWYRQFPKQSLMLMATSNEGSKATYEQGVEKDKFLINHASLTLSTLTVTSAHPEDSSFYICSACSAREQGPLEEQYFGPGTRLTVTEDLRNVTPPKVSLFEPSKAEIANKQKATLVCLARGFFPDHVELSWWVNGKEVHSGVCTDPQAYKESNYSYCLSSRLRVSATFWHNPRNHFRCQVQFHGLSEEDKWPEGSPKPVTQNISAEAWGRADCGITSASYQQGVLSATILYEILLGKATLYAVLVSTLVVMAMVKRKNS

SEQ ID NO: 41 - protein, 7 aa, synthetic construct
  REGION 1..7: note = Description of Artificial Sequence: Synthetic peptide
TISGNEY

SEQ ID NO: 42 - protein, 5 aa, synthetic construct
  REGION 1..5: note = Description of Artificial Sequence: Synthetic peptide
GLKNN

SEQ ID NO: 43 - protein, 14 aa, synthetic construct
  REGION 1..14: note = Description of Artificial Sequence: Synthetic peptide
CIVRVAGSARQLTF

SEQ ID NO: 44 - protein, 5 aa, synthetic construct
  REGION 1..5: note = Description of Artificial Sequence: Synthetic peptide
SGHDT

SEQ ID NO: 45 - protein, 6 aa, synthetic construct
  REGION 1..6: note = Description of Artificial Sequence: Synthetic peptide
YYEEEE

SEQ ID NO: 46 - protein, 14 aa, synthetic construct
  REGION 1..14: note = Description of Artificial Sequence: Synthetic peptide
CASSFGTATYEQYF

SEQ ID NO: 47 - protein, 128 aa, synthetic construct
  REGION 1..128: note = Description of Artificial Sequence: Synthetic polypeptide
MRLVARVTVFLTFGTIIDAKTTQPPSMDCAEGRAANLPCNHSTISGNEYVYWYRQIHSQGPQYIIHGLKNNETNEMASLIITEDRKSSTLILPHATLRDTAVYYCIVRVAGSARQLTFGSGTQLTVLP

SEQ ID NO: 48 - protein, 132 aa, synthetic construct
  REGION 1..132: note = Description of Artificial Sequence: Synthetic polypeptide
MGPGLLCWALLCLLGAGLVDAGVTQSPTHLIKTRGQQVTLRCSPKSGHDTVSWYQQALGQGPQFIFQYYEEEERQRGNFPDRFSGHQFPNYSSELNVNALLLGDSALYLCASSFGTATYEQYFGPGTRLTVT

SEQ ID NO: 49 - protein, 265 aa, synthetic construct
  REGION 1..265: note = Description of Artificial Sequence: Synthetic polypeptide
MRLVARVTVFLTFGTIIDAKTTQPPSMDCAEGRAANLPCNHSTISGNEYVYWYRQIHSQGPQYIIHGLKNNETNEMASLIITEDRKSSTLILPHATLRDTAVYYCIVRVAGSARQLTFGSGTQLTVLPNIQNPEPAVYQLKDPRSQDSTLCLFTDFDSQINVPKTMESGTFITDKCVLDMKAMDSKSNGAIAWSNQTSFTCQDIFKETNATYPSSDVPCDATLTEKSFETDMNLNFQNLLVIVLRILLLKVAGFNLLMTLRLWSS

SEQ ID NO: 50 - protein, 305 aa, synthetic construct
  REGION 1..305: note = Description of Artificial Sequence: Synthetic polypeptide
MGPGLLCWALLCLLGAGLVDAGVTQSPTHLIKTRGQQVTLRCSPKSGHDTVSWYQQALGQGPQFIFQYYEEEERQRGNFPDRFSGHQFPNYSSELNVNALLLGDSALYLCASSFGTATYEQYFGPGTRLTVTEDLRNVTPPKVSLFEPSKAEIANKQKATLVCLARGFFPDHVELSWWVNGKEVHSGVCTDPQAYKESNYSYCLSSRLRVSATFWHNPRNHFRCQVQFHGLSEEDKWPEGSPKPVTQNISAEAWGRADCGITSASYQQGVLSATILYEILLGKATLYAVLVSTLVVMAMVKRKNS

SEQ ID NO: 51 - protein, 6 aa, synthetic construct
  REGION 1..6: note = Description of Artificial Sequence: Synthetic peptide
DSASNY

SEQ ID NO: 52 - protein, 7 aa, synthetic construct
  REGION 1..7: note = Description of Artificial Sequence: Synthetic peptide
IRSNVGE

SEQ ID NO: 53 - protein, 14 aa, synthetic construct
  REGION 1..14: note = Description of Artificial Sequence: Synthetic peptide
CAASIPGTASKLTF

SEQ ID NO: 54 - protein, 5 aa, synthetic construct
  REGION 1..5: note = Description of Artificial Sequence: Synthetic peptide
MNHEY

SEQ ID NO: 55 - protein, 6 aa, synthetic construct
  REGION 1..6: note = Description of Artificial Sequence: Synthetic peptide
SMNVEV

SEQ ID NO: 56 - protein, 15 aa, synthetic construct
  REGION 1..15: note = Description of Artificial Sequence: Synthetic peptide
CASSPYRQGSYGYTF

SEQ ID NO: 57 - protein, 132 aa, synthetic construct
  REGION 1..132: note = Description of Artificial Sequence: Synthetic polypeptide
MTSIRAVFIFLWLQLDLVNGENVEQHPSTLSVQEGDSAVIKCTYSDSASNYFPWYKQELGKGPQLIIDIRSNVGEKKDQRIAVTLNKTAKHFSLHITETQPEDSAVYFCAASIPGTASKLTFGTGTRLQVTL

SEQ ID NO: 58 - protein, 133 aa, synthetic construct
  REGION 1..133: note = Description of Artificial Sequence: Synthetic polypeptide
MGPQLLGYVVLCLLGAGPLEAQVTQNPRYLITVTGKKLTVTCSQNMNHEYMSWYRQDPGLGLRQIYYSMNVEVTDKGDVPEGYKVSRKEKRNFPLILESPSPNQTSLYFCASSPYRQGSYGYTFGSGTRLTVV

SEQ ID NO: 59 - protein, 269 aa, synthetic construct
  REGION 1..269: note = Description of Artificial Sequence: Synthetic polypeptide
MTSIRAVFIFLWLQLDLVNGENVEQHPSTLSVQEGDSAVIKCTYSDSASNYFPWYKQELGKGPQLIIDIRSNVGEKKDQRIAVTLNKTAKHFSLHITETQPEDSAVYFCAASIPGTASKLTFGTGTRLQVTLNIQNPEPAVYQLKDPRSQDSTLCLFTDFDSQINVPKTMESGTFITDKCVLDMKAMDSKSNGAIAWSNQTSFTCQDIFKETNATYPSSDVPCDATLTEKSFETDMNLNFQNLLVIVLRILLLKVAGFNLLMTLRLWSS

SEQ ID NO: 60 - protein, 306 aa, synthetic construct
  REGION 1..306: note = Description of Artificial Sequence: Synthetic polypeptide
MGPQLLGYVVLCLLGAGPLEAQVTQNPRYLITVTGKKLTVTCSQNMNHEYMSWYRQDPGLGLRQIYYSMNVEVTDKGDVPEGYKVSRKEKRNFPLILESPSPNQTSLYFCASSPYRQGSYGYTFGSGTRLTVVEDLRNVTPPKVSLFEPSKAEIANKQKATLVCLARGFFPDHVELSWWVNGKEVHSGVCTDPQAYKESNYSYCLSSRLRVSATFWHNPRNHFRCQVQFHGLSEEDKWPEGSPKPVTQNISAEAWGRADCGITSASYQQGVLSATILYEILLGKATLYAVLVSTLVVMAMVKRKNS

SEQ ID NO: 61 - protein, 6 aa, synthetic construct
  REGION 1..6: note = Description of Artificial Sequence: Synthetic peptide
NTAFDY

SEQ ID NO: 62 - protein, 7 aa, synthetic construct
  REGION 1..7: note = Description of Artificial Sequence: Synthetic peptide
IRPDVSE

SEQ ID NO: 63 - protein, 13 aa, synthetic construct
  REGION 1..13: note = Description of Artificial Sequence: Synthetic peptide
CAASTGNFNKFYF

SEQ ID NO: 64 - protein, 5 aa, synthetic construct
  REGION 1..5: note = Description of Artificial Sequence: Synthetic peptide
SGHNS

SEQ ID NO: 65 - protein, 6 aa, synthetic construct
  REGION 1..6: note = Description of Artificial Sequence: Synthetic peptide
FNNNVP

SEQ ID NO: 66 - protein, 14 aa, synthetic construct
  REGION 1..14: note = Description of Artificial Sequence: Synthetic peptide
CASNRQGTVTEAFF

SEQ ID NO: 67 - protein, 140 aa, synthetic construct
  REGION 1..140: note = Description of Artificial Sequence: Synthetic polypeptide
MDKILGASFLVLWLQLCWVSGQQKEKSDQQQVKQSPQSLIVQKGGISIINCAYENTAFDYFPWYQQFPGKGPALLIAIRPDVSEKKEGRFTISFNKSAKQFSLHIMDSQPGDSATYFCAASTGNFNKFYFGSGTKLNVKP

SEQ ID NO: 68 - protein, 133 aa, synthetic construct
  REGION 1..133: note = Description of Artificial Sequence: Synthetic polypeptide
MDSWTFCCVSLCILVAKHTDAGVIQSPRHEVTEMGQEVTLRCKPISGHNSLFWYRQTMMRGLELLIYFNNNVPIDDSGMPEDRFSAKMPNASFSTLKIQPSEPRDSAVYFCASNRQGTVTEAFFGQGTRLTVV

SEQ ID NO: 69 - protein, 277 aa, synthetic construct
  REGION 1..277: note = Description of Artificial Sequence: Synthetic polypeptide
MDKILGASFLVLWLQLCWVSGQQKEKSDQQQVKQSPQSLIVQKGGISIINCAYENTAFDYFPWYQQFPGKGPALLIAIRPDVSEKKEGRFTISFNKSAKQFSLHIMDSQPGDSATYFCAASTGNFNKFYFGSGTKLNVKPNIQNPEPAVYQLKDPRSQDSTLCLFTDFDSQINVPKTMESGTFITDKCVLDMKAMDSKSNGAIAWSNQTSFTCQDIFKETNATYPSSDVPCDATLTEKSFETDMNLNFQNLLVIVLRILLLKVAGFNLLMTLRLWSS

SEQ ID NO: 70 - protein, 306 aa, synthetic construct
  REGION 1..306: note = Description of Artificial Sequence: Synthetic polypeptide
MDSWTFCCVSLCILVAKHTDAGVIQSPRHEVTEMGQEVTLRCKPISGHNSLFWYRQTMMRGLELLIYFNNNVPIDDSGMPEDRFSAKMPNASFSTLKIQPSEPRDSAVYFCASNRQGTVTEAFFGQGTRLTVVEDLRNVTPPKVSLFEPSKAEIANKQKATLVCLARGFFPDHVELSWWVNGKEVHSGVCTDPQAYKESNYSYCLSSRLRVSATFWHNPRNHFRCQVQFHGLSEEDKWPEGSPKPVTQNISAEAWGRADCGITSASYQQGVLSATILYEILLGKATLYAVLVSTLVVMAMVKRKNS

SEQ ID NO: 71 - protein, 65 aa, synthetic construct
  REGION 1..65: note = Description of Artificial Sequence: Synthetic polypeptide
HAGLSNRLARDNELRENDKEQLKAISTRDPLSEITEQEKDFLWSHRHYCVTIPEILPKLLLSVKW

SEQ ID NO: 72 - protein, 65 aa, synthetic construct
  REGION 1..65: note = Description of Artificial Sequence: Synthetic polypeptide
HAGLSNRLARDNELRENDKEQLKAISTRDPLSKITEQEKDFLWSHRHYCVTIPEILPKLLLSVKW

SEQ ID NO: 73 - protein, 65 aa, synthetic construct
  REGION 1..65: note = Description of Artificial Sequence: Synthetic polypeptide
LSNRLARDNELRENDKEQLKAISTRDPLSEITEQEKDFLWSHRHYCVTIPEILPKLLLSVKWNSR

SEQ ID NO: 74 - protein, 65 aa, synthetic construct
  REGION 1..65: note = Description of Artificial Sequence: Synthetic polypeptide
LSNRLARDNELRENDKEQLKAISTRDPLSEITKQEKDFLWSHRHYCVTIPEILPKLLLSVKWNSR

SEQ ID NO: 75 - protein, 45 aa, synthetic construct
  REGION 1..45: note = Description of Artificial Sequence: Synthetic polypeptide
KTLALDKTEQEALEYFMKQMNDAHHGGWTTKMDWIFHTIKQHALN

SEQ ID NO: 76 - protein, 45 aa, synthetic construct
  REGION 1..45: note = Description of Artificial Sequence: Synthetic polypeptide
KTLALDKTEQEALEYFMKQMNDARHGGWTTKMDWIFHTIKQHALN

SEQ ID NO: 77 - protein, 45 aa, synthetic construct
  REGION 1..45: note = Description of Artificial Sequence: Synthetic polypeptide
KTLALDKTEQEALEYFMKQMNDALHGGWTTKMDWIFHTIKQHALN

SEQ ID NO: 78 - protein, 25 aa, synthetic construct
  REGION 1..25: note = Description of Artificial Sequence: Synthetic peptide
GHSYTTAEELAGIGILTVILGVLLL

SEQ ID NO: 79 - protein, 25 aa, synthetic construct
  REGION 1..25: note = Description of Artificial Sequence: Synthetic peptide
ILGDPKKLLTQHFVQENYLEYRQVP

SEQ ID NO: 80 - protein, 141 aa, Homo sapiens
NIQNPDPAVYQLRDSKSSDKSVCLFTDFDSQTNVSQSKDSDVYITDKTVLDMRSMDFKSNSAVAWSNKSDFACANAFNNSIIPEDTFFPSPESSCDVKLVEKSFETDTNLNFQNLSVIGFRILLLKVAGFNLLMTLRLWSS

SEQ ID NO: 81 - protein, 137 aa, synthetic construct
  REGION 1..137: note = Description of Artificial Sequence: Synthetic polypeptide
NIQNPEPAVYQLKDPRSQDSTLCLFTDFDSQINVPKTMESGTFITDKCVLDMKAMDSKSNGAIAWSNQTSFTCQDIFKETNATYPSSDVPCDATLTEKSFETDMNLNFQNLLVIVLRILLLKVAGFNLLMTLRLWSS

SEQ ID NO: 82 - protein, 177 aa, Homo sapiens
EDLNKVFPPEVAVFEPSEAEISHTQKATLVCLATGFFPDHVELSWWVNGKEVHSGVSTDPQPLKEQPALNDSRYCLSSRLRVSATFWQNPRNHFRCQVQFYGLSENDEWTQDRAKPVTQIVSAEAWGRADCGFTSVSYQQGVLSATILYEILLGKATLYAVLVSALVLMAMVKRKDF

SEQ ID NO: 83 - protein, 173 aa, synthetic construct
  REGION 1..173: note = Description of Artificial Sequence: Synthetic polypeptide
EDLRNVTPPKVSLFEPSKAEIANKQKATLVCLARGFFPDHVELSWWVNGKEVHSGVCTDPQAYKESNYSYCLSSRLRVSATFWHNPRNHFRCQVQFHGLSEEDKWPEGSPKPVTQNISAEAWGRADCGITSASYQQGVLSATILYEILLGKATLYAVLVSTLVVMAMVKRKNS

SEQ ID NO: 84 - protein, 27 aa, unidentified
  REGION 1..27: note = Description of Unknown: Furin-2A-peptide sequence
RAKRSGSGATNFSLLKQAGDVEENPGP

SEQ ID NO: 85 - protein, 4 aa, synthetic construct
  REGION 1..4: note = Description of Artificial Sequence: Synthetic peptide
SGSG

SEQ ID NO: 86 - protein, 15 aa, synthetic construct
  REGION 1..15: note = Description of Artificial Sequence: Synthetic peptide
CAVRPLYGGSYIPTF

SEQ ID NO: 87 - protein, 12 aa, synthetic construct
  REGION 1..12: note = Description of Artificial Sequence: Synthetic peptide
CAVNFGGGKLIF

SEQ ID NO: 88 - protein, 13 aa, synthetic construct
  REGION 1..13: note = Description of Artificial Sequence: Synthetic peptide
CVLGGGSARQLTF

SEQ ID NO: 89 - protein, 13 aa, synthetic construct
  REGION 1..13: note = Description of Artificial Sequence: Synthetic peptide
CAVNKRSNYQLIW

SEQ ID NO: 90 - protein, 12 aa, synthetic construct
  REGION 1..12: note = Description of Artificial Sequence: Synthetic peptide
CVVNDGTYKYIF

SEQ ID NO: 91 - protein, 11 aa, synthetic construct
  REGION 1..11: note = Description of Artificial Sequence: Synthetic peptide
CAASMIARLMF

SEQ ID NO: 92 - protein, 15 aa, synthetic construct
  REGION 1..15: note = Description of Artificial Sequence: Synthetic peptide
CAMRDFSGGYNKLIF

SEQ ID NO: 93 - protein, 11 aa, synthetic construct
  REGION 1..11: note = Description of Artificial Sequence: Synthetic peptide
CAGHPLNDMRF

SEQ ID NO: 94 - protein, 13 aa, synthetic construct
  REGION 1..13: note = Description of Artificial Sequence: Synthetic peptide
CAFVRNNNARLMF

SEQ ID NO: 95 - protein, 15 aa, synthetic construct
  REGION 1..15: note = Description of Artificial Sequence: Synthetic peptide
CAESLMDTGRRALTF

SEQ ID NO: 96 - protein, 14 aa, synthetic construct
  REGION 1..14: note = Description of Artificial Sequence: Synthetic peptide
CASSYVGNTGELFF

SEQ ID NO: 97 - protein, 13 aa, synthetic construct
  REGION 1..13: note = Description of Artificial Sequence: Synthetic peptide
CASSLSFGTEAFF

SEQ ID NO: 98 - protein, 12 aa, synthetic construct
  REGION 1..12: note = Description of Artificial Sequence: Synthetic peptide
CASSRMNTEAFF

SEQ ID NO: 99 - protein, 14 aa, synthetic construct
  REGION 1..14: note = Description of Artificial Sequence: Synthetic peptide
CASSYFQGAAEAFF

SEQ ID NO: 100 - protein, 13 aa, synthetic construct
  REGION 1..13: note = Description of Artificial Sequence: Synthetic peptide
CASSPKQQYEQYF

SEQ ID NO: 101 - protein, 15 aa, synthetic construct
  REGION 1..15: note = Description of Artificial Sequence: Synthetic peptide
CASSFTTGVGTEAFF

SEQ ID NO: 102 - protein, 12 aa, synthetic construct
  REGION 1..12: note = Description of Artificial Sequence: Synthetic peptide
CASRKQNYGYTF

SEQ ID NO: 103 - protein, 14 aa, synthetic construct
  REGION 1..14: note = Description of Artificial Sequence: Synthetic peptide
CASSENGGVDEQFF

SEQ ID NO: 104 - protein, 17 aa, synthetic construct
  REGION 1..17: note = Description of Artificial Sequence: Synthetic peptide
CASSSAFTGTEDPGYTF

SEQ ID NO: 105 - protein, 15 aa, synthetic construct
  REGION 1..15: note = Description of Artificial Sequence: Synthetic peptide
CASSEWTSGDNEQFF

SEQ ID NO: 106 - protein, 15 aa, synthetic construct
  REGION 1..15: note = Description of Artificial Sequence: Synthetic peptide
CASSLGTFSTDTQYF

SEQ ID NO: 107 - protein, 15 aa, synthetic construct
  REGION 1..15: note = Description of Artificial Sequence: Synthetic peptide
CASSQGGRGEYEAFF

SEQ ID NO: 108 - protein, 11 aa, synthetic construct
  REGION 1..11: note = Description of Artificial Sequence: Synthetic peptide
CASSPGYEQFF

SEQ ID NO: 109 - protein, 20 aa, synthetic construct
  REGION 1..20: note = Description of Artificial Sequence: Synthetic peptide
CASSHPLGGQGNTWGNEQFF

SEQ ID NO: 110 - protein, 12 aa, synthetic construct
  REGION 1..12: note = Description of Artificial Sequence: Synthetic peptide
CASSFSGTGAFF

SEQ ID NO: 111 - protein, 15 aa, synthetic construct
  REGION 1..15: note = Description of Artificial Sequence: Synthetic peptide
CASSPTGTSGNEQYF

SEQ ID NO: 112 - protein, 14 aa, synthetic construct
  REGION 1..14: note = Description of Artificial Sequence: Synthetic peptide
CASSEGHLNTEAFF

SEQ ID NO: 113 - protein, 12 aa, synthetic construct
  REGION 1..12: note = Description of Artificial Sequence: Synthetic peptide
CASSRVQNEQFF

SEQ ID NO: 114 - protein, 15 aa, synthetic construct
  REGION 1..15: note = Description of Artificial Sequence: Synthetic peptide
CASSFSGTPPQPQHF

SEQ ID NO: 115 - protein, 13 aa, synthetic construct
  REGION 1..13: note = Description of Artificial Sequence: Synthetic peptide
CASSLQGYNEQFF

SEQ ID NO: 116 - protein, 13 aa, synthetic construct
  REGION 1..13: note = Description of Artificial Sequence: Synthetic peptide
CASSIPGKETQYF

SEQ ID NO: 117 - protein, 14 aa, synthetic construct
  REGION 1..14: note = Description of Artificial Sequence: Synthetic peptide
CASSTTLTGIKDTF

SEQ ID NO: 118 - protein, 13 aa, synthetic construct
  REGION 1..13: note = Description of Artificial Sequence: Synthetic peptide
CASSYGLTYEQYF

SEQ ID NO: 119 - protein, 16 aa, synthetic construct
  REGION 1..16: note = Description of Artificial Sequence: Synthetic peptide
CASSSLGDVMNTEAFF

SEQ ID NO: 120 - protein, 13 aa, synthetic construct
  REGION 1..13: note = Description of Artificial Sequence: Synthetic peptide
CASSRGLQPTQYF

SEQ ID NO: 121 - protein, 13 aa, synthetic construct
  REGION 1..13: note = Description of Artificial Sequence: Synthetic peptide
CASSFNPSYEQYF

SEQ ID NO: 122 - protein, 15 aa, synthetic construct
  REGION 1..15: note = Description of Artificial Sequence: Synthetic peptide
CASSLSGGGDYGYTF

SEQ ID NO: 123 - protein, 14 aa, synthetic construct
  REGION 1..14: note = Description of Artificial Sequence: Synthetic peptide
CASGGSGNTGKLIF

SEQ ID NO: 124 - protein, 14 aa, synthetic construct
  REGION 1..14: note = Description of Artificial Sequence: Synthetic peptide
CASSLGQFNYEQYF

SEQ ID NO: 125 - protein, 606 aa, synthetic construct
  REGION 1..606: note = Description of Artificial Sequence: Synthetic polypeptide
MDTRVLCCAVICLLGAGLSNAGVMQNPRHLVRRRGQEARLRCSPMKGHSHVYWYRQLPEEGLKFMVYLQKENIIDESGMPKERFSAEFPKEGPSILRIQQVVRGDSAAYFCASSPVNLAGVSRADTQYFGPGTRLTVLEDLRNVTPPKVSLFEPSKAEIANKQKATLVCLARGFFPDHVELSWWVNGKEVHSGVCTDPQAYKESNYSYCLSSRLRVSATFWHNPRNHFRCQVQFHGLSEEDKWPEGSPKPVTQNISAEAWGRADCGITSASYQQGVLSATILYEILLGKATLYAVLVSTLVVMAMVKRKNSRAKRSGSGATNFSLLKQAGDVEENPGPMETLLGLLILWLQLQWVSSKQEVTQIPAALSVPEGENLVLNCSFTDSAIYNLQWFRQDPGKGLTSLLLIQSSQREQTSGRLNASLDKSSGRSTLYIAASQPGDSATYLCAVKGSDDYKLSFGAGTTVTVRANIQNPEPAVYQLKDPRSQDSTLCLFTDFDSQINVPKTMESGTFITDKCVLDMKAMDSKSNGAIAWSNQTSFTCQDIFKETNATYPSSDVPCDATLTEKSFETDMNLNFQNLLVIVLRILLLKVAGFNLLMTLRLWSS

SEQ ID NO: 126 - protein, 598 aa, synthetic construct
  REGION 1..598: note = Description of Artificial Sequence: Synthetic polypeptide
MGTRLLFWVAFCLLGAYHTGAGVSQSPSNKVTEKGKDVELRCDPISGHTALYWYRQRLGQGLEFLIYFQGNSAPDKSGLPSDRFSAERTGESVSTLTIQRTQQEDSAVYLCASSPRGYQPQHFGDGTRLSILEDLRNVTPPKVSLFEPSKAEIANKQKATLVCLARGFFPDHVELSWWVNGKEVHSGVCTDPQAYKESNYSYCLSSRLRVSATFWHNPRNHFRCQVQFHGLSEEDKWPEGSPKPVTQNISAEAWGRADCGITSASYQQGVLSATILYEILLGKATLYAVLVSTLVVMAMVKRKNSRAKRSGSGATNFSLLKQAGDVEENPGPMWGVFLLYVSMKMGGTTGQNIDQPTEMTATEGAIVQINCTYQTSGFNGLFWYQQHAGEAPTFLSYNVLDGLEEKGRFSSFLSRSKGYSYLLLKELQMKDSASYLCAVTSWGKLQFKLQFGAGTQVVVTPNIQNPEPAVYQLKDPRSQDSTLCLFTDFDSQINVPKTMESGTFITDKCVLDMKAMDSKSNGAIAWSNQTSFTCQDIFKETNATYPSSDVPCDATLTEKSFETDMNLNFQNLLVIVLRILLLKVAGFNLLMTLRLWSS

SEQ ID NO: 127 - protein, 608 aa, synthetic construct
  REGION 1..608: note = Description of Artificial Sequence: Synthetic polypeptide
MDTRVLCCAVICLLGAGLSNAGVMQNPRHLVRRRGQEARLRCSPMKGHSHVYWYRQLPEEGLKFMVYLQKENIIDESGMPKERFSAEFPKEGPSILRIQQVVRGDSAAYFCASSPPEAGLDTEAFFGQGTRLTVVEDLRNVTPPKVSLFEPSKAEIANKQKATLVCLARGFFPDHVELSWWVNGKEVHSGVCTDPQAYKESNYSYCLSSRLRVSATFWHNPRNHFRCQVQFHGLSEEDKWPEGSPKPVTQNISAEAWGRADCGITSASYQQGVLSATILYEILLGKATLYAVLVSTLVVMAMVKRKNSRAKRSGSGATNFSLLKQAGDVEENPGPMSLSSLLKVVTASLWLGPGIAQKITQTQPGMFVQEKEAVTLDCTYDTSDQSYGLFWYKQPSSGEMIFLIYQGSYDEQNATEGRYSLNFQKARKSANLVISASQLGDSAMYFCAMREVLDNTDKLIFGTGTRLQVFPNIQNPEPAVYQLKDPRSQDSTLCLFTDFDSQINVPKTMESGTFITDKCVLDMKAMDSKSNGAIAWSNQTSFTCQDIFKETNATYPSSDVPCDATLTEKSFETDMNLNFQNLLVIVLRILLLKVAGFNLLMTLRLWSS

SEQ ID NO: 128 - protein, 604 aa, synthetic construct
  REGION 1..604: note = Description of Artificial Sequence: Synthetic polypeptide
MLLLLLLLGPAGSGLGAVVSQHPSRVICKSGTSVKIECRSLDFQATTMFWYRQFPKQSLMLMATSNEGSKATYEQGVEKDKFLINHASLTLSTLTVTSAHPEDSSFYICSACSAREQGPLEEQYFGPGTRLTVTEDLRNVTPPKVSLFEPSKAEIANKQKATLVCLARGFFPDHVELSWWVNGKEVHSGVCTDPQAYKESNYSYCLSSRLRVSATFWHNPRNHFRCQVQFHGLSEEDKWPEGSPKPVTQNISAEAWGRADCGITSASYQQGVLSATILYEILLGKATLYAVLVSTLVVMAMVKRKNSRAKRSGSGATNFSLLKQAGDVEENPGPMMKSLRVLLVILWLQLSWVWSQQKEVEQDPGPLSVPEGAIVSLNCTYSNSAFQYFMWYRQYSRKGPELLMYTYSSGNKEDGRFTAQVDKSSKYISLFIRDSQPSDSATYLCAMNSGGYQKVTFGIGTKLQVIPNIQNPEPAVYQLKDPRSQDSTLCLFTDFDSQINVPKTMESGTFITDKCVLDMKAMDSKSNGAIAWSNQTSFTCQDIFKETNATYPSSDVPCDATLTEKSFETDMNLNFQNLLVIVLRILLLKVAGFNLLMTLRLWSS

SEQ ID NO: 129 - protein, 597 aa, synthetic construct
  REGION 1..597: note = Description of Artificial Sequence: Synthetic polypeptide
MGPGLLCWALLCLLGAGLVDAGVTQSPTHLIKTRGQQVTLRCSPKSGHDTVSWYQQALGQGPQFIFQYYEEEERQRGNFPDRFSGHQFPNYSSELNVNALLLGDSALYLCASSFGTATYEQYFGPGTRLTVTEDLRNVTPPKVSLFEPSKAEIANKQKATLVCLARGFFPDHVELSWWVNGKEVHSGVCTDPQAYKESNYSYCLSSRLRVSATFWHNPRNHFRCQVQFHGLSEEDKWPEGSPKPVTQNISAEAWGRADCGITSASYQQGVLSATILYEILLGKATLYAVLVSTLVVMAMVKRKNSRAKRSGSGATNFSLLKQAGDVEENPGPMRLVARVTVFLTFGTIIDAKTTQPPSMDCAEGRAANLPCNHSTISGNEYVYWYRQIHSQGPQYIIHGLKNNETNEMASLIITEDRKSSTLILPHATLRDTAVYYCIVRVAGSARQLTFGSGTQLTVLPNIQNPEPAVYQLKDPRSQDSTLCLFTDFDSQINVPKTMESGTFITDKCVLDMKAMDSKSNGAIAWSNQTSFTCQDIFKETNATYPSSDVPCDATLTEKSFETDMNLNFQNLLVIVLRILLLKVAGFNLLMTLRLWSS

SEQ ID NO: 130 - protein, 602 aa, synthetic construct
  REGION 1..602: note = Description of Artificial Sequence: Synthetic polypeptide
MGPQLLGYVVLCLLGAGPLEAQVTQNPRYLITVTGKKLTVTCSQNMNHEYMSWYRQDPGLGLRQIYYSMNVEVTDKGDVPEGYKVSRKEKRNFPLILESPSPNQTSLYFCASSPYRQGSYGYTFGSGTRLTVVEDLRNVTPPKVSLFEPSKAEIANKQKATLVCLARGFFPDHVELSWWVNGKEVHSGVCTDPQAYKESNYSYCLSSRLRVSATFWHNPRNHFRCQVQFHGLSEEDKWPEGSPKPVTQNISAEAWGRADCGITSASYQQGVLSATILYEILLGKATLYAVLVSTLVVMAMVKRKNSRAKRSGSGATNFSLLKQAGDVEENPGPMTSIRAVFIFLWLQLDLVNGENVEQHPSTLSVQEGDSAVIKCTYSDSASNYFPWYKQELGKGPQLIIDIRSNVGEKKDQRIAVTLNKTAKHFSLHITETQPEDSAVYFCAASIPGTASKLTFGTGTRLQVTLNIQNPEPAVYQLKDPRSQDSTLCLFTDFDSQINVPKTMESGTFITDKCVLDMKAMDSKSNGAIAWSNQTSFTCQDIFKETNATYPSSDVPCDATLTEKSFETDMNLNFQNLLVIVLRILLLKVAGFNLLMTLRLWSS

SEQ ID NO: 131 - protein, 610 aa, synthetic construct
  REGION 1..610: note = Description of Artificial Sequence: Synthetic polypeptide
MDSWTFCCVSLCILVAKHTDAGVIQSPRHEVTEMGQEVTLRCKPISGHNSLFWYRQTMMRGLELLIYFNNNVPIDDSGMPEDRFSAKMPNASFSTLKIQPSEPRDSAVYFCASNRQGTVTEAFFGQGTRLTVVEDLRNVTPPKVSLFEPSKAEIANKQKATLVCLARGFFPDHVELSWWVNGKEVHSGVCTDPQAYKESNYSYCLSSRLRVSATFWHNPRNHFRCQVQFHGLSEEDKWPEGSPKPVTQNISAEAWGRADCGITSASYQQGVLSATILYEILLGKATLYAVLVSTLVVMAMVKRKNSRAKRSGSGATNFSLLKQAGDVEENPGPMDKILGASFLVLWLQLCWVSGQQKEKSDQQQVKQSPQSLIVQKGGISIINCAYENTAFDYFPWYQQFPGKGPALLIAIRPDVSEKKEGRFTISFNKSAKQFSLHIMDSQPGDSATYFCAASTGNFNKFYFGSGTKLNVKPNIQNPEPAVYQLKDPRSQDSTLCLFTDFDSQINVPKTMESGTFITDKCVLDMKAMDSKSNGAIAWSNQTSFTCQDIFKETNATYPSSDVPCDATLTEKSFETDMNLNFQNLLVIVLRILLLKVAGFNLLMTLRLWSS